European Patent Specification EP 3 710 001 B1, published June 18, 2025. Title: COMPOUNDS AND METHODS FOR REGULATING, LIMITING, OR INHIBITING AVIL EXPRESSION. Applicant: University of Virginia Patent Foundation. The sequence listing filed with the application follows.

SEQUENCE LISTING (9 sequences)

SEQ ID NO: 1 - DNA, 3687 bp, Homo sapiens
atgagactgttcgtgagtgatggcgtcccgggttgcttgccggtgctggccgccgccgggagagcccggggcagagcagaggtgctcatcagcactgtaggcccggaagattgtgtggtcccgttcctgacccggcctaaggtccctgtcttgcagctggatagcggcaactacctcttctccactagtgcaatctgccgatatttttttttgttatctggctgggagcaagatgacctcactaaccagtggctggaatgggaagcgacagagctgcagccagctttgtctgctgccctgtactatttagtggtccaaggcaagaagggggaagatgttcttggttcagtgcggagagccctgactcacattgaccacagcttgagtcgtcagaactgtcctttcctggctggggagacagaatctctagccgacattgttttgtggggagccctatacccattactgcaagatcccgcctacctccctgaggagctgagtgccctgcacagctggttccagacactgagtacccaggaaccatgtcagcgagctgcagagactgtactgaaacagcaaggtgtcctggctctccggccttacctccaaaagcagccccagcccagccccgctgagggaagggctgtcaccaatgagcctgaggaggaggagctggctaccctatctgaggaggagattgctatggctgttactgcttgggagaagggcctagaaagtttgcccccgctgcggccccagcagaatccagtgttgcctgtggctggagaaaggaatgtgctcatcaccagtgccctcccttacgtcaacaatgtcccccaccttgggaacatcattggttgtgtgctcagtgccgatgtctttgccaggtactctcgcctccgccagtggaacaccctctatctgtgtgggacagatgagtatggtacagcaacagagaccaaggctctggaggagggactaaccccccaggagatctgcgacaagtaccacatcatccatgctgacatctaccgctggtttaacatttcgtttgatatttttggtcgcaccaccactccacagcagaccaaaatcacccaggacattttccagcagttgctgaaacgaggttttgtgctgcaagatactgtggagcaactgcgatgtgagcactgtgctcgcttcctggctgaccgcttcgtggagggcgtgtgtcccttctgtggctatgaggaggctcggggtgaccagtgtgacaagtgtggcaagctcatcaatgctgtcgagcttaagaaaatggagctggcgctggtgcctgtgagcgcccacggcaacttctatgagggggactgctacgtcatcctctcgacccggagagtggccagtctcctatcccaggacatccacttctggatcgggaaggactcctcccaggatgagcaaagctgcgcagccatatataccacacagctggacgactacctgggaggcagccctgtgcagcaccgagaggtccagtaccatgagtcagacactttccgtggctacttcaagcagggcatcatctacaagcaggggggtgtcgcctctgggatgaagcacgtggagaccaatacctacgacgtgaagcggctgctacatgtgaaagggaaaagaaacatcagggctaccgaggtggaaatgagctgggacagtttcaaccgaggtgatgtcttcttgctggaccttgggaaagtcatcatccaatggaatggcccagagagcaacagtggggagcgcctgaaggctatgcttctggcaaaggatattcgagacagggagcgagggggccgtgctaaaataggagtgatcgagggagacaaggaggcagccagcccagagctgatgaaggtccttcaggacacccttggccgacgctccattatcaagcctacagtccctgatgagatcatagatcagaagcagaaatcaactatcatgttgtatcatatctcagattcagctgggcagctggcagtcacagaggtagcaacaaggcctctggtccaggacttactgaaccatgatgactgctacatcctggaccaaagtggaaccaaaatctacgtgtggaaaggaaaaggagccacaaaggctgaaaaacaggcagccatgtctaaagcgctgggcttcatcaagatgaagagctaccccagcagcaccaatgtggagaccgtcaacgatggtgctgagtcggccatgttcaagcagctgttccagaagtggtcagtaaaggaccagaccatgggcctggggaaaacgttcagcattggtaaaattgctaaagttttccaggataaatttgatgtgactctgctacacaccaagccagaggtagctgcccaggaaagaatggtcgatgatggcaacggaaaagttgaggtctggagaattgagaacctggagctggtccctgtggagtatcaatggtatggcttcttttatgggggagactgttatctggtcctctacacatacgaggtaaatgggaagccacatcacatcttgtacatctggcagggccgccacgcctcacaggatgagctggcagcctcagcataccaggcagtggaggtggatcggcagtttgatggggctgctgtgcaggttcgagtcaggatgggaacggagccacgccacttcatggccatcttcaaagggaagctagttatctttgagggtgggacttccaggaagggaaatgccgagcctgaccctccagtaagactcttccaaattcatggaaatgacaaatctaacaccaaagcagtggaagttccagcctttgcctcctccctaaactccaatgatgtctttctgctgcgaactcaggcagagcactacctgtggtatggcaaggggtctagtggggatgagcgggcaatggctaaggagctggccagccttctctgtgatggcagcgagaacactgtggccgagggccaggagccagccgagttctgggacctactgggagggaaaactccctatgccaatgataaaagacttcagcaggaaatcctagatgtccagtctcgtctctttgaatgttccaataagaccggccaattcgttgtcactgagatcacagacttcacccaggatgacctgaaccctactgacgtgatgctcctagatacctgggaccaggtgttcttgtggattggggctgaggccaatgccacggagaaggagagtgcccttgccacagcacagcagtacctgcacactcaccccagcggccgagatcccgacacaccaatcctgatcattaagcaggggtttgagcctcccatcttcacaggctggttcctagcctgggaccctaacatttggagtgcaggaaaaacatatgaacaattaaaagaagagctgggagatgctgctgctatcatgcgaatcactgctgacatgaagaatgcaaccctctccctgaattctaatgacagtgagccaaaatattaccctatagcagttctgttgaaaaaccagaatcaggagctgcctgaggatgtaaaccctgccaaaaaggagaattacctctctgaacaggactttgtgtctgtgtttggcatcacaagagggcaatttgcagctctgcctggctggaaacagctccaaatgaagaaagaaaaggggcttttctaa

SEQ ID NO: 2 - DNA, 2460 bp, Homo sapiens
atgcctctgaccagtgccttcagggctgtggacaacgaccctgggatcattgtctggagaatagagaaaatggagctggcgctggtgcctgtgagcgcccacggcaacttctatgagggggactgctacgtcatcctctcgacccggagagtggccagtctcctatcccaggacatccacttctggatcgggaaggactcctcccaggatgagcaaagctgcgcagccatatataccacacagctggacgactacctgggaggcagccctgtgcagcaccgagaggtccagtaccatgagtcagacactttccgtggctacttcaagcagggcatcatctacaagcaggggggtgtcgcctctgggatgaagcacgtggagaccaatacctacgacgtgaagcggctgctacatgtgaaagggaaaagaaacatcagggctaccgaggtggaaatgagctgggacagtttcaaccgaggtgatgtcttcttgctggaccttgggaaagtcatcatccaatggaatggcccagagagcaacagtggggagcgcctgaaggctatgcttctggcaaaggatattcgagacagggagcgagggggccgtgctaaaataggagtgatcgagggagacaaggaggcagccagcccagagctgatgaaggtccttcaggacacccttggccgacgctccattatcaagcctacagtccctgatgagatcatagatcagaagcagaaatcaactatcatgttgtatcatatctcagattcagctgggcagctggcagtcacagaggtagcaacaaggcctctggtccaggacttactgaaccatgatgactgctacatcctggaccaaagtggaaccaaaatctacgtgtggaaaggaaaaggagccacaaaggctgaaaaacaggcagccatgtctaaagcgctgggcttcatcaagatgaagagctaccccagcagcaccaatgtggagaccgtcaacgatggtgctgagtcggccatgttcaagcagctgttccagaagtggtcagtaaaggaccagaccatgggcctggggaaaacgttcagcattggtaaaattgctaaagttttccaggataaatttgatgtgactctgctacacaccaagccagaggtagctgcccaggaaagaatggtcgatgatggcaacggaaaagttgaggtctggagaattgagaacctggagctggtccctgtggagtatcaatggtatggcttcttttatgggggagactgttatctggtcctctacacatacgaggtaaatgggaagccacatcacatcttgtacatctggcagggccgccacgcctcacaggatgagctggcagcctcagcataccaggcagtggaggtggatcggcagtttgatggggctgctgtgcaggttcgagtcaggatgggaacggagccacgccacttcatggccatcttcaaagggaagctagttatctttgagggtgggacttccaggaagggaaatgccgagcctgaccctccagtaagactcttccaaattcatggaaatgacaaatctaacaccaaagcagtggaagttccagcctttgcctcctccctaaactccaatgatgtctttctgctgcgaactcaggcagagcactacctgtggtatggcaaggggtctagtggggatgagcgggcaatggctaaggagctggccagccttctctgtgatggcagcgagaacactgtggccgagggccaggagccagccgagttctgggacctactgggagggaaaactccctatgccaatgataaaagacttcagcaggaaatcctagatgtccagtctcgtctctttgaatgttccaataagaccggccaattcgttgtcactgagatcacagacttcacccaggatgacctgaaccctactgacgtgatgctcctagatacctgggaccaggtgttcttgtggattggggctgaggccaatgccacggagaaggagagtgcccttgccacagcacagcagtacctgcacactcaccccagcggccgagatcccgacacaccaatcctgatcattaagcaggggtttgagcctcccatcttcacaggctggttcctagcctgggaccctaacatttggagtgcaggaaaaacatatgaacaattaaaagaagagctgggagatgctgctgctatcatgcgaatcactgctgacatgaagaatgcaaccctctccctgaattctaatgacagtgagccaaaatattaccctatagcagttctgttgaaaaaccagaatcaggagctgcctgaggatgtaaaccctgccaaaaaggagaattacctctctgaacaggactttgtgtctgtgtttggcatcacaagagggcaatttgcagctctgcctggctggaaacagctccaaatgaagaaagaaaaggggcttttctaa

SEQ ID NO: 3 - RNA, 19 nt, Artificial Sequence
  Synthetic Construct
gcuucuggcaaaggauauu

SEQ ID NO: 4 - RNA, 19 nt, Artificial Sequence
  Synthetic Construct
ccacacagcuggacgacua

SEQ ID NO: 5 - RNA, 19 nt, Artificial Sequence
  Synthetic Construct
gcaaaggauauucgagaca

SEQ ID NO: 6 - RNA, 19 nt, Artificial Sequence
  Synthetic Construct
gcaccaauguggagaccgu

SEQ ID NO: 7 - RNA, 19 nt, Artificial Sequence
  Synthetic Construct
ggaaagaauggucgaugau

SEQ ID NO: 8 - RNA, 19 nt, Artificial Sequence
  Synthetic Construct
gcauuccuugcuuguuaua

SEQ ID NO: 9 - RNA, 19 nt, Artificial Sequence
  Synthetic Construct
gagcuuaagaaaauggagc